European Patent Specification EP 3 576 789 B1, published December 11, 2024. Title: Monomeric Human IgG1 Fc And Bispecific Antibodies. Applicant: SMET Pharmaceutical Inc. CHEN, Weizao XIAO, Zuoxiang FU, Tao. Application PCT/US18/16524. The sequence listing filed with the application follows.

SEQUENCE LISTING (34 sequences)

SEQ ID NO: 1 - protein, 217 aa, Homo sapiens
APELLGGPSVFLFPPKPKDTLMISRTPEVTCVVVDVSHEDPEVKFNWYVDGVEVHNAKTKPREEQYNSTYRVVSVLTVLHQDWLNGKEYKCKVSNKALPAPIEKTISKAKGQPREPQVYTLPPSRDELTKNQVSLTCLVKGFYPSDIAVEWESNGQPENNYKTTPPVLDSDGSFFLYSKLTVDKSRWQQGNVFSCSVMHEALHNHYTQKSLSLSPGK

SEQ ID NO: 2 - protein, 217 aa, Artificial Sequence
  human IgG1 with mutants
APELLGGPSVFLFPPKPKDTLMISRTPEVTCVVVDVSHEDPEVKFNWYVDGVEVHNAKTKPREEQYNSTYRVVSVLTVLHQDWLNGKEYKCKVSNKALPAPIEKTISKAKGQPREPQVYTLPPSRDELTKNQVSLDCLVKGFYPSDIAVEWESNGQPENNYKTTPPVLDSDGSFFLISKLTVDKSRWQQGNVFSCSVMHEALHNHYTQKSLSLSPGK

SEQ ID NO: 3 - protein, 217 aa, Artificial Sequence
  human IgG1 with mutants
APELLGGPSVFLFPPKPKDTLMISRTPEVTCVVVDVSHEDPEVKFNWYVDGVEVHNAKTKPREEQYNSTYRVVSVLTVLHQDWLNGKEYKCKVSNKALPAPIEKTISKAKGQPREPQVYTLPPSRDELTKNQVSLLCLVKGFYPSDIAVEWESNGQPENNYKTTPPVLDSDGSFFLFSKLTVDKSRWQQGNVFSCSVMHEALHNHYTQKSLSLSPGK

SEQ ID NO: 4 - protein, 217 aa, Artificial Sequence
  human IgG1 with mutants
APELLGGPSVFLFPPKPKDTLMISRTPEVTCVVVDVSHEDPEVKFNWYVDGVEVHNAKTKPREEQYNSTYRVVSVLTVLHQDWLNGKEYKCKVSNKALPAPIEKTISKAKGQPREPQVYTLPPSRDELTKNQVSLTCLVKGFYPSDIAVEWESNGQPENNYKTTPPVLDSDGSFFLLSKLTVDKSRWQQGNVFSCSVMHEALHNHYTQKSLSLSPGK

SEQ ID NO: 5 - protein, 217 aa, Artificial Sequence
  human IgG1 with mutants
APELLGGPSVFLFPPKPKDTLMISRTPEVTCVVVDVSHEDPEVKFNWYVDGVEVHNAKTKPREEQYNSTYRVVSVLTVLHQDWLNGKEYKCKVSNKALPAPIEKTISKAKGQPREPQVYTLPPSRDELTKNQVSLLCLVKGFYPSDIAVEWESNGQPENNYKTTPPVLDSDGSFFLMSKLTVDKSRWQQGNVFSCSVMHEALHNHYTQKSLSLSPGK

SEQ ID NO: 6 - protein, 217 aa, Artificial Sequence
  human IgG1 with mutants
APELLGGPSVFLFPPKPKDTLMISRTPEVTCVVVDVSHEDPEVKFNWYVDGVEVHNAKTKPREEQYNSTYRVVSVLTVLHQDWLNGKEYKCKVSNKALPAPIEKTISKAKGQPREPQVYTLPPSRDELTKNQVSLLCLVKGFYPSDIAVEWESNGQPENNYKTTPPVLDSDGSFFLYSKLTVDKSRWQQGNVFSCSVMHEALHNHYTQKSLSLSPGK

SEQ ID NO: 7 - protein, 217 aa, Artificial Sequence
  human IgG1 with mutants
APELLGGPSVFLFPPKPKDTLMISRTPEVTCVVVDVSHEDPEVKFNWYVDGVEVHNAKTKPREEQYNSTYRVVSVLTVLHQDWLNGKEYKCKVSNKALPAPIEKTISKAKGQPREPQVYTLPPSRDELTKNQVSLWCLVKGFYPSDIAVEWESNGQPENNYKTTPPVLDSDGSFFLFSKLTVDKSRWQQGNVFSCSVMHEALHNHYTQKSLSLSPGK

SEQ ID NO: 8 - protein, 217 aa, Artificial Sequence
  human IgG1 with mutants
APELLGGPSVFLFPPKPKDTLMISRTPEVTCVVVDVSHEDPEVKFNWYVDGVEVHNAKTKPREEQYNSTYRVVSVLTVLHQDWLNGKEYKCKVSNKALPAPIEKTISKAKGQPREPQVYTLPPSRDELTKNQVSLNCLVKGFYPSDIAVEWESNGQPENNYKTTPPVLDSDGSFFLLSKLTVDKSRWQQGNVFSCSVMHEALHNHYTQKSLSLSPGK

SEQ ID NO: 9 - protein, 217 aa, Artificial Sequence
  human IgG1 with mutants
APELLGGPSVFLFPPKPKDTLMISRTPEVTCVVVDVSHEDPEVKFNWYVDGVEVHNAKTKPREEQYNSTYRVVSVLTVLHQDWLNGKEYKCKVSNKALPAPIEKTISKAKGQPREPQVYTLPPSRDELTKNQVSLLCLVKGFYPSDIAVEWESNGQPENNYKTTPPVLDSDGSFFLHSKLTVDKSRWQQGNVFSCSVMHEALHNHYTQKSLSLSPGK

SEQ ID NO: 10 - protein, 217 aa, Artificial Sequence
  human IgG1 with mutants
APELLGGPSVFLFPPKPKDTLMISRTPEVTCVVVDVSHEDPEVKFNWYVDGVEVHNAKTKPREEQYNSTYRVVSVLTVLHQDWLNGKEYKCKVSNKALPAPIEKTISKAKGQPREPQVYTLPPSRDELTKNQVSLLCLVKGFYPSDIAVEWESNGQPENNYKTTPPVLDSDGSFFLKSKLTVDKSRWQQGNVFSCSVMHEALHNHYTQKSLSLSPGK

SEQ ID NO: 11 - protein, 217 aa, Artificial Sequence
  human IgG1 with mutants
APELLGGPSVFLFPPKPKDTLMISRTPEVTCVVVDVSHEDPEVKFNWYVDGVEVHNAKTKPREEQYNSTYRVVSVLTVLHQDWLNGKEYKCKVSNKALPAPIEKTISKAKGQPREPQVYTLPPSRDELTKNQVSLLCLVKGFYPSDIAVEWESNGQPENNYKTTPPVLDSDGSFFLSSKLTVDKSRWQQGNVFSCSVMHEALHNHYTQKSLSLSPGK

SEQ ID NO: 12 - protein, 217 aa, Artificial Sequence
  human IgG1 with mutants
APELLGGPSVFLFPPKPKDTLMISRTPEVTCVVVDVSHEDPEVKFNWYVDGVEVHNAKTKPREEQYNSTYRVVSVLTVLHQDWLNGKEYKCKVSNKALPAPIEKTISKAKGQPREPQVYTLPPSRDELTKNQVSLLCLVKGFYPSDIAVEWESNGQPENNYKTTPPVLDSDGSFFLQSKLTVDKSRWQQGNVFSCSVMHEALHNHYTQKSLSLSPGK

SEQ ID NO: 13 - protein, 217 aa, Artificial Sequence
  human IgG1 with mutants
APELLGGPSVFLFPPKPKDTLMISRTPEVTCVVVDVSHEDPEVKFNWYVDGVEVHNAKTKPREEQYNSTYRVVSVLTVLHQDWLNGKEYKCKVSNKALPAPIEKTISKAKGQPREPQVYTLPPSRDELTKNQVSLLCLVKGFYPSDIAVEWESNGQPENNYKTTPPVLDSDGSFFLTSKLTVDKSRWQQGNVFSCSVMHEALHNHYTQKSLSLSPGK

SEQ ID NO: 14 - protein, 217 aa, Artificial Sequence
  human IgG1 with mutants
APELLGGPSVFLFPPKPKDTLMISRTPEVTCVVVDVSHEDPEVKFNWYVDGVEVHNAKTKPREEQYNSTYRVVSVLTVLHQDWLNGKEYKCKVSNKALPAPIEKTISKAKGQPREPQVYTLPPSRDELTKNQVSLLCLVKGFYPSDIAVEWESNGQPENNYKTTPPVLDSDGSFFLWSKLTVDKSRWQQGNVFSCSVMHEALHNHYTQKSLSLSPGK

SEQ ID NO: 15 - protein, 217 aa, Artificial Sequence
  human IgG1 with mutants
APELLGGPSVFLFPPKPKDTLMISRTPEVTCVVVDVSHEDPEVKFNWYVDGVEVHNAKTKPREEQYNSTYRVVSVLTVLHQDWLNGKEYKCKVSNKALPAPIEKTISKAKGQPREPQVYTLPPSRDELTKNQVSLLCLVKGFYPSDIAVEWESNGQPENNYKTTPPVLDSDGSFFLASKLTVDKSRWQQGNVFSCSVMHEALHNHYTQKSLSLSPGK

SEQ ID NO: 16 - protein, 217 aa, Artificial Sequence
  human IgG1 with mutants
APELLGGPSVFLFPPKPKDTLMISRTPEVTCVVVDVSHEDPEVKFNWYVDGVEVHNAKTKPREEQYNSTYRVVSVLTVLHQDWLNGKEYKCKVSNKALPAPIEKTISKAKGQPREPQVYTLPPSRDELTKNQVSLLCLVKGFYPSDIAVEWESNGQPENNYKTTPPVLDSDGSFFLGSKLTVDKSRWQQGNVFSCSVMHEALHNHYTQKSLSLSPGK

SEQ ID NO: 17 - protein, 217 aa, Artificial Sequence
  human IgG1 with mutants
APELLGGPSVFLFPPKPKDTLMISRTPEVTCVVVDVSHEDPEVKFNWYVDGVEVHNAKTKPREEQYNSTYRVVSVLTVLHQDWLNGKEYKCKVSNKALPAPIEKTISKAKGQPREPQVYTLPPSRDELTKNQVSLLCLVKGFYPSDIAVEWESNGQPENNYKTTPPVLDSDGSFFLNSKLTVDKSRWQQGNVFSCSVMHEALHNHYTQKSLSLSPGK

SEQ ID NO: 18 - DNA, 35 bp, Artificial Sequence
  Oligo primer
gatcggcccaggcggccgcacctgaactcctgggg

SEQ ID NO: 19 - DNA, 20 bp, Artificial Sequence
  Oligo primer
caggctgacctggttcttgg

SEQ ID NO: 20 - DNA, 33 bp, Artificial Sequence
  Oligo primer
  misc_feature (13)..(14): "n" means "a" or "g" or "c" or "t"
caggtcagcctgnnstgcctggtcaaaggcttc

SEQ ID NO: 21 - DNA, 18 bp, Artificial Sequence
  Oligo primer
gaggaagaaggagccgtc

SEQ ID NO: 22 - DNA, 36 bp, Artificial Sequence
  Oligo primer
  misc_feature (16)..(17): "n" means "a" or "g" or "c" or "t"
ggctccttcttcctcnnsagcaagctcaccgtggac

SEQ ID NO: 23 - DNA, 34 bp, Artificial Sequence
  Oligo primer
gatcggccggcctggcctttacccggagacaggg

SEQ ID NO: 24 - DNA, 33 bp, Artificial Sequence
  Oligo primer
  misc_feature (16)..(17): "n" means "a" or "g" or "c" or "t"
ggctccttcttcctcnnsagcaagctcaccgtg

SEQ ID NO: 25 - DNA, 18 bp, Artificial Sequence
  Oligo primer
gaggaagaaggagccgtc

SEQ ID NO: 26 - DNA, 46 bp, Artificial Sequence
  Oligo primer
gtgtaagcttaccatgggtgtgcccactcaggtcctggggttgctg

SEQ ID NO: 27 - DNA, 32 bp, Artificial Sequence
  Oligo primer
tgggcacggtggacactctcccctgttgaagc

SEQ ID NO: 28 - DNA, 33 bp, Artificial Sequence
  Oligo primer
tgtccaccgtgcccagcacctgaactcctgggg

SEQ ID NO: 29 - DNA, 30 bp, Artificial Sequence
  Oligo primer
gatcgaattcttatttacccggagacaggg

SEQ ID NO: 30 - DNA, 46 bp, Artificial Sequence
  Oligo primer
gtgttctagagccgccaccatggaatggagctgggtctttctcttc

SEQ ID NO: 31 - DNA, 30 bp, Artificial Sequence
  Oligo primer
tgggcacggtggacaagatttgggctcaac

SEQ ID NO: 32 - DNA, 32 bp, Artificial Sequence
  Oligo primer
cggccgtcgcactcatttacccggagacaggg

SEQ ID NO: 33 - DNA, 18 bp, Artificial Sequence
  Oligo primer
tgagtgcgacggccggca

SEQ ID NO: 34 - DNA, 18 bp, Artificial Sequence
  Oligo primer
cccgaggtcgacgctctc